European Patent Application EP 4 733 408 A2, published April 29, 2026. Title: METHODS TO MINIMIZE BARCODE EXCHANGE. Applicant: 10X GENOMICS, INC. Application EP, filed August 2, 2019. The sequence listing filed with the application follows.

SEQUENCE LISTING (9 sequences)

SEQ ID NO: 1 - DNA, 312 bp, synthetic construct
  misc_feature 1..312: note = Description of Artificial Sequence: Synthetic polynucleotide
  source 1..312: mol_type = other DNA
aatgatacggcgaccaccgagatctacacgactagtgtacccacgtcgtcggcagcgtcagatgtgtataagagacagatgggtagctctcaccatcatcatcatcactctagcggtctggtccctcgcggtagccacatgccacgtaaaatgtatagctgtgattttgagactacgacgaaagttgaagattgccgtgtgtgggcgtatggttacatgaatattgaagatcactccgagtataagattggcaatagcctggatgaattcatggcgtgctgtctcttatacacatctccgagcccacgagac

SEQ ID NO: 2 - DNA, 312 bp, synthetic construct
  misc_feature 1..312: note = Description of Artificial Sequence: Synthetic polynucleotide
  source 1..312: mol_type = other DNA
aatgatacggcgaccaccgagatctacacatctgaagacatcgtctcgtcggcagcgtcagatgtgtataagagacagatgggtagctctcaccatcatcatcatcactctagcggtctggtccctcgcggtagccacatgccacgtaaaatgtatagctgtgattttgagactacgacgaaagttgaagattgccgtgtgtgggcgtatggttacatgaatattgaagatcactccgagtataagattggcaatagcctggatgaattcatggcgtgctgtctcttatacacatctccgagcccacgagac

SEQ ID NO: 3 - DNA, 312 bp, synthetic construct
  misc_feature 1..312: note = Description of Artificial Sequence: Synthetic polynucleotide
  source 1..312: mol_type = other DNA
aatgatacggcgaccaccgagatctacactcagcgtcttccatgatcgtcggcagcgtcagatgtgtataagagacagatgggtagctctcaccatcatcatcatcactctagcggtctggtccctcgcggtagccacatgccacgtaaaatgtatagctgtgattttgagactacgacgaaagttgaagattgccgtgtgtgggcgtatggttacatgaatattgaagatcactccgagtataagattggcaatagcctggatgaattcatggcgtgctgtctcttatacacatctccgagcccacgagac

SEQ ID NO: 4 - DNA, 312 bp, synthetic construct
  misc_feature 1..312: note = Description of Artificial Sequence: Synthetic polynucleotide
  source 1..312: mol_type = other DNA
aatgatacggcgaccaccgagatctacaccgtatcctcaggtcagtcgtcggcagcgtcagatgtgtataagagacagatgggtagctctcaccatcatcatcatcactctagcggtctggtccctcgcggtagccacatgccacgtaaaatgtatagctgtgattttgagactacgacgaaagttgaagattgccgtgtgtgggcgtatggttacatgaatattgaagatcactccgagtataagattggcaatagcctggatgaattcatggcgtgctgtctcttatacacatctccgagcccacgagac

SEQ ID NO: 5 - DNA, 45 bp, synthetic construct
  misc_feature 1..45: note = Description of Artificial Sequence: Synthetic oligonucleotide
  source 1..45: mol_type = other DNA
aatgatacggcgaccaccgagatctacacgagcatgaggtagact

SEQ ID NO: 6 - DNA, 59 bp, synthetic construct
  misc_feature 1..59: note = Description of Artificial Sequence: Synthetic oligonucleotide
  source 1..59: mol_type = other DNA
gacgctgccgacgaagtctacctcatgctcgtgtagatctcggtggtcgccgtatcatt

SEQ ID NO: 7 - DNA, 59 bp, synthetic construct
  misc_feature 1..59: note = Description of Artificial Sequence: Synthetic oligonucleotide
  misc_feature 1..59: note = Description of Combined DNA/RNA Molecule: Synthetic oligonucleotide
  source 1..59: mol_type = other DNA
  modified_base 10: mod_base = OTHER; note = uracil
gacgctgcctacgaagtctacctcatgctcgtgtagatctcggtggtcgccgtatcatt

SEQ ID NO: 8 - DNA, 59 bp, synthetic construct
  modified_base 10: mod_base = OTHER; note = Abasic "idSp" nucleotide
  misc_feature 1..59: note = Description of Artificial Sequence: Synthetic oligonucleotide
  source 1..59: mol_type = other DNA
gacgctgccnacgaagtctacctcatgctcgtgtagatctcggtggtcgccgtatcatt

SEQ ID NO: 9 - DNA, 78 bp, synthetic construct
  misc_difference 30..36: note = a, c, t, g, unknown or other
  misc_difference 39..45: note = a, c, t, g, unknown or other
  misc_feature 1..78: note = Description of Artificial Sequence: Synthetic oligonucleotide
  misc_feature 1..78: note = Description of Combined DNA/RNA Molecule: Synthetic oligonucleotide
  source 1..78: mol_type = other DNA
aatgatacggcgaccaccgagatctacacnnnnnnngtnnnnnnntcgtcggcagcgtcagatgtgtataagagacaa